European Patent Specification EP 3 446 707 B1, published August 5, 2026. Title: SURROGATE BINDING PROTEINS. Applicant: Arun K. Kashyap Ramesh R. Bhatt Michael Horowitz Lawrence Horowitz Sihong Zhou Ryann E. O'Neil. The sequence listing filed with the application follows.

SEQUENCE LISTING (501 sequences)

SEQ ID NO: 1 - protein, 145 aa, Homo sapiens
MSWAPVLLMLFVYCTGCGPQPVLHQPPAMSSALGTTIRLTCTLRNDHDIGVYSVYWYQQRPGHPPRFLLRYFSQSDKSQGPQVPPRFSGSKDVARNRGYLSISELQPEDEAMYYCAMGARSSEKEEREREWEEEMEPTAARTRVP

SEQ ID NO: 2 - protein, 142 aa, Mus musculus
MAWTSVLLMLLAHLTGCGPQPMVHQPPSASSSLGATIRLSCTLSNDHNIGIYSIYWYQQRPGHPPRFLLRYFSHSDKHQGPDIPPRFSGSKDTARNLGYLSISELQPEDEAVYYCAVGLRSHEKKRMEREWEGEKSYTDLGS

SEQ ID NO: 3 - protein, 171 aa, Mus musculus
MAWTSVLLMLLAHLTGKGTLGVQGFLAPPVALLCPSDGHASIFSGCGPQPMVHQPPSASSSLGATIRLSCTLSNDHNIGIYSIYWYQQRPGHPPRFLLRYFSHSDKHQGPDIPPRFSGSKDTARNLGYLSISELQPEDEAVYYCAVGLRSHEKKRMEREWEGEKSYTDLGS

SEQ ID NO: 4 - protein, 123 aa, Homo sapiens
MACRCLSFLLMGTFLSVSQTVLAQLDALLVFPGQVAQLSCTLSPQHVTIRDYGVSWYQQRAGSAPRYLLYYRSEEDHHRPADIPDRFSAAKDEAHNACVLTISPVQPEDDADYYCSVGYGFSP

SEQ ID NO: 5 - protein, 209 aa, Mus musculus
MKLRVGQTLGTIPRQCEVLLLLLLLGLVDGVHHILSPSSAERSRAVGPGASVGSNRPSLWALPGRLLFQIIPRGAGPRCSPHRLPSKPQFWYVFGGGTQLTILGQPKSDPLVTLFLPSLKNLQPTRPHVVCLVSEFYPGTLVVDWKVDGVPVTQGVETTQPSKQTNNKYMVSSYLTLISDQWMPHSRYSCRVTHEGNTVEKSVSPAECS

SEQ ID NO: 6 - protein, 213 aa, Homo sapiens
MRPGTGQGGLEAPGEPGPNLRQRWPLLLLGLAVVTHGLLRPTAASQSRALGPGAPGGSSRSSLRSRWGRFLLQRGSWTGPRCWPRGFQSKHNSVTHVFGSGTQLTVLSQPKATPSVTLFPPSSEELQANKATLVCLMNDFYPGILTVTWKADGTPITQGVEMTTPSKQSNNKYAASSYLSLTPEQWRSRRSYSCQVMHEGSTVEKTVAPAECS

SEQ ID NO: 7 - protein, 158 aa, Artificial Sequence
  Synthetic Construct
MRPGTGQGGLEAPGEPGPNLRQRWPLLLLGLAVVTHGSVTHVFGSGTQLTVLSQPKATPSVTLFPPSSEELQANKATLVCLMNDFYPGILTVTWKADGTPITQGVEMTTPSKQSNNKYAASSYLSLTPEQWRSRRSYSCQVMHEGSTVEKTVAPAECS

SEQ ID NO: 8-9 - skipped (2 entries)

SEQ ID NO: 10 - protein, 242 aa, Artificial Sequence
  Synthetic Construct
MSWAPVLLMLFVYCTGCGPQPVLHQPPAMSSALGTTIRLTCTLRNDHDIGVYSVYWYQQRPGHPPRFLLRYFSQSDKSQGPQVPPRFSGSKDVARNRGYLSISELQPEDEAMYYCAMGARSSVTHVFGSGTQLTVLSQPKATPSVTLFPPSSEELQANKATLVCLMNDFYPGILTVTWKADGTPITQGVEMTTPSKQSNNKYAASSYLSLTPEQWRSRRSYSCQVMHEGSTVEKTVAPAECS

SEQ ID NO: 11 - protein, 243 aa, Artificial Sequence
  Synthetic Construct
METDTLLLWVLLLWVPGSTGQPVLHQPPAMSSALGTTIRLTCTLRNDHDIGVYSVYWYQQRPGHPPRFLLRYFSQSDKSQGPQVPPRFSGSKDVARNRGYLSISELQPEDEAMYYCAMGARSSVTHVFGGGTKLTVLSQPKAAPSVTLFPPSSEELQANTATLVCLISDFYPGAVTVAWKADSSPVKAGVETTTPSKQSNNKYAASSYLSLTPEQWKSHRSYSCQVTHEGSTVEKTVAPTECS

SEQ ID NO: 12 - protein, 256 aa, Artificial Sequence [sequence omitted]

SEQ ID NO: 13 - protein, 135 aa, Artificial Sequence
  Synthetic Construct
AQPVLHQPPAMSSALGTTIRLTCTLRNDHDIGVYSVYWYQQRPGHPPRFLLRYFSQSDKSQGPQVPPRFSGSKDVARNRGYLSISELQPEDEAMYYCAMGARSSEKERLPSKPQFWYVFGGGTQLTILGQPKSDP

SEQ ID NO: 14 - protein, 104 aa, Homo sapiens
QAVLTQPASLSASPGASASLTCTLRSGINVGTYRIYWYQQKPGSPPQYLLRYKSDSDKQQGSGVPSRFSGSKDASANAGILLISGLQSEDEADYYCMIWHSSAS

SEQ ID NO: 15 - protein, 105 aa, Homo sapiens
QPVLTQPSSHSASSGASVRLTCMLSSGFSVGDFWIRWYQQKPGNPPRYLLYYHSDSNKGQGSGVPSRFSGSNDASANAGILRISGLQPEDEADYYCGTWHSNSKT

SEQ ID NO: 16 - protein, 104 aa, Homo sapiens
QPVLTQPPSSSASPGESARLTCTLPSDINVGSYNIYWYQQKPGSPPRYLLYYYSDSDKGQGSGVPSRFSGSKDASANTGILLISGLQSEDEADYYCMIWPSNAS

SEQ ID NO: 17 - protein, 113 aa, Homo sapiens
GTKLTVLRQPKAAPSVTLFPPSSEELQANKATLVCLISDFYPGAVTVAWKADGSPVKAGVETTTPSKQSNNKYAASSYLSLTPEQWKSHKSYSCQVTHEGSTVEKTVAPTECS

SEQ ID NO: 18 - protein, 213 aa, Homo sapiens; identical to SEQ ID NO: 6

SEQ ID NO: 19 - protein, 213 aa, Homo sapiens; identical to SEQ ID NO: 6

SEQ ID NO: 20 - protein, 107 aa, Homo sapiens [sequence omitted]

SEQ ID NO: 21 - protein, 159 aa, Homo sapiens
MARIPKTLKFVVVIVAVLLPVLAYSATTARQEEVPQQTVAPQQQRHSFKGEECPAGSHRSEHTGACNPCTEGVDYTNASNNEPSCFPCTVCKSDQKHKSSCTMTRDTVCQCKEGTFRNENSPEMCRKCSRCPSGEVQVSNCTSWDDIQCVEEFGANATV

SEQ ID NO: 22 - protein, 238 aa, Homo sapiens
APPPARVHLGAFLAVTPNPGSAASGTEAAAATPSKVWGSSAGRIEPRGGGRGALPTSMGQHGPSARARAGRAPGPRPAREASPRLRVHKTFKFVVVGVLLQVVPSSAATIKLHDQSIGTQQWEHSPLGELCPPGSHRSEHPGACNRCTEGVGYTNASNNLFACLPCTACKSDEEERSPCTTTRNTACQCKPGTFRNDNSAEMCRKCSRGCPRGMVKVKDCTPWSDIECVHKESGNGHN

SEQ ID NO: 23 - protein, 189 aa, Homo sapiens
MGLWGQSVPTASSARAGRYPGARTASGTRPWLLDPKILKFVVFIVAVLLPVRVDSATIPRQDEVPQQTVAPQQQRRSLKEEECPAGSHRSEYTGACNPCTEGVDYTIASNNLPSCLLCTVCKSGQTNKSSCTTTRDTVCQCEKGSFQDKNSPEMCRTCRTGCPRGMVKVSNCTPRSDIKCKNESAASST

SEQ ID NO: 24 - protein, 188 aa, Homo sapiens
MEQRGQNAPAASGARKRHGPGPREARGARPGLRVPKTLVLVVAAVLLLVSAESALITQQDLAPQQRVAPQQKRSSPSEGLCPPGHHISEDGRDCISCKYGQDYSTHWNDLLFCLRCTRCDSGEVELSPCTTTRNTVCQCEEGTFREEDSPEMCRKCRTGCPRGMVKVGDCTPWSDIECVHKESGTKHS

SEQ ID NO: 25 - protein, 132 aa, Homo sapiens
AATIKLHDQSIGTQQWEHSPLGELCPPGSHRSEHPGACNRCTEGVGYTNASNNLFACLPCTACKSDEEERSPCTTTRNTACQCKPGTFRNDNSAEMCRKCSRGCPRGMVKVKDCTPWSDIECVHKESGNGHN

SEQ ID NO: 26 - protein, 135 aa, Homo sapiens
ALITQQDLAPQQRVAPQQKRSSPSEGLCPPGHHISEDGRDCISCKYGQDYSTHWNDLLFCLRCTRCDSGEVELSPCTTTRNTVCQCEEGTFREEDSPEMCRKCRTGCPRGMVKVGDCTPWSDIECVHKESGTKHS

SEQ ID NO: 27 - protein, 133 aa, Mus musculus
FVPVTANPAHNRPAGLQRPEESPSRGPCLAGQYLSEGNCKPCREGIDYTSHSNHSLDSCILCTVCKEDKVVETRCNITTNTVCRCKPGTFEDKDSPEICQSCSNCTDGEEELTSCTPRENRKCVSKTAWASWH

SEQ ID NO: 28-37 - skipped (10 entries)

SEQ ID NO: 38 - protein, 121 aa, Homo sapiens
EVQLVESGGGLVKPGGSLRLSCAASGFTFSTYGMHWVRQAPGKGLEWVAGINYSGNNKYYADSVKGRFTISRDNAKNSLYLQMNSLRAEDTAVYYCARDHSTWLSRHLDYWGQGTLVTVSS

SEQ ID NO: 39 - protein, 6 aa, Homo sapiens
STYGMH

SEQ ID NO: 40 - protein, 13 aa, Homo sapiens
WVAGINYSGNNKY

SEQ ID NO: 41 - protein, 13 aa, Homo sapiens
ARDHSTWLSRHLD

SEQ ID NO: 42 - protein, 117 aa, Homo sapiens
EVQLVESGGGLVKPGGSLRLSCAASGFTFSSYAMSWVRQAPGKGLEWVSSISSSSSYIYYADSVKGRFTISRDNAKNSLYLQMNSLRAEDTAVYYCARSFGGPYVYWGQGTLVTVSS

SEQ ID NO: 43 - protein, 6 aa, Homo sapiens
SSYAMS

SEQ ID NO: 44 - protein, 13 aa, Homo sapiens
WVSSISSSSSYIY

SEQ ID NO: 45 - protein, 9 aa, Homo sapiens
ARSFGGPYV

SEQ ID NO: 46 - protein, 117 aa, Homo sapiens
EVQLLESGGGLVQPGGSLRLSCAASGFTFRSYAMNWVRQAPGKGLEWVALISYDSSYIYYADSVKGRFTISRDNSKNTLYLQMNSLRAEDTAVYYCARLLRGGFDYWGQGTLVTVSS

SEQ ID NO: 47 - protein, 6 aa, Homo sapiens
RSYAMN

SEQ ID NO: 48 - protein, 13 aa, Homo sapiens
WVALISYDSSYIY

SEQ ID NO: 49 - protein, 9 aa, Homo sapiens
ARLLRGGFD

SEQ ID NO: 50 - protein, 117 aa, Homo sapiens
EVQLLESGGGLVQPGGSLRLSCAASGFTFRSFAMSWVRQAPGKGLEWVATISAGGGYINYADSVKGRFTISRDNSKNTLYLQMNSLRAEDTAVYYCARVQSWVLDYWGQGTLVTVSS

SEQ ID NO: 51 - protein, 6 aa, Homo sapiens
RSFAMS

SEQ ID NO: 52 - protein, 13 aa, Homo sapiens
WVATISAGGGYIN

SEQ ID NO: 53 - protein, 9 aa, Homo sapiens
ARVQSWVLD

SEQ ID NO: 54 - protein, 117 aa, Homo sapiens
EVQLVESGGGLVKPGGSLRLSCAASGFTFSSYAMSWVRQAPGKGLEWVASIGYDGSYKYYADSVKGRFTISRDNAKNSLYLQMNSLRAEDTAVYYCARGVSRGYVYWGQGTLVTVSS

SEQ ID NO: 55 - protein, 6 aa, Homo sapiens
SSYAMS

SEQ ID NO: 56 - protein, 13 aa, Homo sapiens
WVASIGYDGSYKY

SEQ ID NO: 57 - protein, 9 aa, Homo sapiens
ARGVSRGYV

SEQ ID NO: 58 - protein, 117 aa, Homo sapiens
QVQLVQSGAEVKKPGASVKVSCKASGYTFSNYAMSWVRQAPGQGLEWMGWITPNSGTAKYAQKFQGRVTMTRDTSISTAYMELSRLRSDDTAVYYCARGVSGYYDYWGQGTLVTVSS

SEQ ID NO: 59 - protein, 6 aa, Homo sapiens
SNYAMS

SEQ ID NO: 60 - protein, 13 aa, Homo sapiens
WMGWITPNSGTAK

SEQ ID NO: 61 - protein, 9 aa, Homo sapiens
ARGVSGYYD

SEQ ID NO: 62 - protein, 117 aa, Homo sapiens
QVQLVQSGAEVKKPGSSVKVSCKASGGTFSAYPISWVRQAPGQGLEWMGWISPGSGNTNYAQKFQGRVTITADKSTSTAYMELSSLRSEDTAVYYCARGVGGYFDYWGQGTLVTVSS

SEQ ID NO: 63 - protein, 6 aa, Homo sapiens
SAYPIS

SEQ ID NO: 64 - protein, 13 aa, Homo sapiens
WMGWISPGSGNTN

SEQ ID NO: 65 - protein, 9 aa, Homo sapiens
ARGVGGYFD

SEQ ID NO: 66 - protein, 117 aa, Homo sapiens
EVQLVESGGGLVKPGGSLRLSCAASGFTFSSYSMNWVRQAPGKGLEWVAAIANDSAYTYYADSVKGRFTISRDNAKNSLYLQMNSLRAEDTAVYYCARGPSSRLVYWGQGTLVTVSS

SEQ ID NO: 67 - protein, 6 aa, Homo sapiens
SSYSMN

SEQ ID NO: 68 - protein, 13 aa, Homo sapiens
WVAAIANDSAYTY

SEQ ID NO: 69 - protein, 9 aa, Homo sapiens
ARGPSSRLV

SEQ ID NO: 70 - protein, 117 aa, Homo sapiens
EVQLVESGGGLVKPGGSLRLSCAASGFTFSSYSMNWVRQAPGKGLEWVAAIANDSAYTYYADSVKGRFTISRDNAKNSLYLQMNSLRAEDTAVYYCARGPSTRLVYWGQGTLVTVSS

SEQ ID NO: 71 - protein, 6 aa, Homo sapiens
SSYSMN

SEQ ID NO: 72 - protein, 13 aa, Homo sapiens
WVAAIANDSAYTY

SEQ ID NO: 73 - protein, 9 aa, Homo sapiens
ARGPSTRLV

SEQ ID NO: 74 - protein, 117 aa, Homo sapiens
EVQLVESGGGLVKPGGSLRLSCAASGFTFRNYAMSWVRQAPGKGLEWVAGINYSGTYTYYADSVKGRFTISRDNAKNSLYLQMNSLRAEDTAVYYCARGFGRGFVYWGQGTLVTVSS

SEQ ID NO: 75 - protein, 6 aa, Homo sapiens
RNYAMS

SEQ ID NO: 76 - protein, 13 aa, Homo sapiens
WVAGINYSGTYTY

SEQ ID NO: 77 - protein, 9 aa, Homo sapiens
ARGFGRGFV

SEQ ID NO: 78 - protein, 117 aa, Homo sapiens
EVQLVESGGGLVKPGGSLRLSCAASGFTFSNYGMSWVRQAPGKGLEWVSSISSSSSYIYYADSVKGRFTISRDNAKNSLYLQMNSLRAEDTAVYYCARGFGRGYVYWGQGTLVTVSS

SEQ ID NO: 79 - protein, 6 aa, Homo sapiens
SNYGMS

SEQ ID NO: 80 - protein, 13 aa, Homo sapiens
WVSSISSSSSYIY

SEQ ID NO: 81 - protein, 9 aa, Homo sapiens
ARGFGRGYV

SEQ ID NO: 82 - protein, 118 aa, Homo sapiens
EVQLLESGGGLVQPGGSLRLSCAASGFTFSSYSMSWVRQAPGKGLEWVAGIGWGGTTKYYADSVKGRFTISRDNSKNTLYLQMNSLRAEDTAVYYCARGGYRAYIDYWGQGTLVTVSS

SEQ ID NO: 83 - protein, 6 aa, Homo sapiens
SSYSMS

SEQ ID NO: 84 - protein, 13 aa, Homo sapiens
WVAGIGWGGTTKY

SEQ ID NO: 85 - protein, 10 aa, Homo sapiens
ARGGYRAYID

SEQ ID NO: 86 - protein, 118 aa, Homo sapiens
QVQLVQSGAEVKKPGASVKVSCKASGYTFTNYYMHWVRQAPGQGLEWMGWINPNSGNTNYAQKFQGRVTMTRDTSISTAYMELSRLRSDDTAVYYCAREVVRYGFDYWGQGTLVTVSS

SEQ ID NO: 87 - protein, 6 aa, Homo sapiens
TNYYMH

SEQ ID NO: 88 - protein, 13 aa, Homo sapiens
WMGWINPNSGNTN

SEQ ID NO: 89 - protein, 10 aa, Homo sapiens
AREVVRYGFD

SEQ ID NO: 90 - protein, 119 aa, Homo sapiens
EVQLVESGGGLVKPGGSLRLSCAASGFTFRNYGMNWVRQAPGKGLEWVAGIKNDGDTKYYADSVKGRFTISRDNAKNSLYLQMNSLRAEDTAVYYCAKRVRYGHAMDYWGQGTLVTVSS

SEQ ID NO: 91 - protein, 6 aa, Homo sapiens
RNYGMN

SEQ ID NO: 92 - protein, 13 aa, Homo sapiens
WVAGIKNDGDTKY

SEQ ID NO: 93 - protein, 11 aa, Homo sapiens
AKRVRYGHAMD

SEQ ID NO: 94 - protein, 119 aa, Homo sapiens
EVQLLESGGGLVQPGGSLRLSCAASGFTFRNFAMNWVRQAPGKGLEWVAGIKYDGSNKYYADSVKGRFTISRDNSKNTLYLQMNSLRAEDTAVYYCARRRWAGHGFDYWGQGTLVTVSS

SEQ ID NO: 95 - protein, 6 aa, Homo sapiens
RNFAMN

SEQ ID NO: 96 - protein, 13 aa, Homo sapiens
WVAGIKYDGSNKY

SEQ ID NO: 97 - protein, 11 aa, Homo sapiens
ARRRWAGHGFD

SEQ ID NO: 98 - protein, 119 aa, Homo sapiens
EVQLLESGGGLVQPGGSLRLSCAASGFTFSNYAMNWVRQAPGKGLEWVSAISGSGGSTYYADSVKGRFTISRDNSKNTLYLQMNSLRAEDTAVYYCARRRWAGHGFDYWGQGTLVTVSS

SEQ ID NO: 99 - protein, 6 aa, Homo sapiens
SNYAMN

SEQ ID NO: 100 - protein, 13 aa, Homo sapiens
WVSAISGSGGSTY

SEQ ID NO: 101 - protein, 11 aa, Homo sapiens
ARRRWAGHGFD

SEQ ID NO: 102 - protein, 119 aa, Homo sapiens
EVQLVESGGGLVKPGGSLRLSCAASGFTFSSYSMNWVRQAPGKGLEWVAAISYNGANKYYADSVKGRFTISRDNAKNSLYLQMNSLRAEDTAVYYCARKVGYPSAFDYWGQGTLVTVSS

SEQ ID NO: 103 - protein, 6 aa, Homo sapiens
SSYSMN

SEQ ID NO: 104 - protein, 13 aa, Homo sapiens
WVAAISYNGANKY

SEQ ID NO: 105 - protein, 11 aa, Homo sapiens
ARKVGYPSAFD

SEQ ID NO: 106 - protein, 119 aa, Homo sapiens
EVQLVESGGGLVKPGGSLRLSCAASGFTFSSYAMSWVRQAPGKGLEWVAAISYGSDYINYADSVKGRFTISRDNAKNSLYLQMNSLRAEDTAVYYCARRYAWGAGMDYWGQGTLVTVSS

SEQ ID NO: 107 - protein, 6 aa, Homo sapiens
SSYAMS

SEQ ID NO: 108 - protein, 13 aa, Homo sapiens
WVAAISYGSDYIN

SEQ ID NO: 109 - protein, 11 aa, Homo sapiens
ARRYAWGAGMD

SEQ ID NO: 110 - protein, 119 aa, Homo sapiens
EVQLVESGGGLVKPGGSLRLSCAASGFTFSSYSMSWVRQAPGKGLEWVASISYGSGYKNYADSVKGRFTISRDNAKNSLYLQMNSLRAEDTAVYYCARRYAGGYGFDYWGQGTLVTVSS

SEQ ID NO: 111 - protein, 6 aa, Homo sapiens
SSYSMS

SEQ ID NO: 112 - protein, 13 aa, Homo sapiens
WVASISYGSGYKN

SEQ ID NO: 113 - protein, 11 aa, Homo sapiens
ARRYAGGYGFD

SEQ ID NO: 114 - protein, 119 aa, Homo sapiens
EVQLLESGGGLVQPGGSLRLSCAASGFTFSSYSMSWVRQAPGKGLEWVSAISYNSANIYYADSVKGRFTISRDNSKNTLYLQMNSLRAEDTAVYYCARRLGWGNGFDYWGQGTLVTVSS

SEQ ID NO: 115 - protein, 6 aa, Homo sapiens
SSYSMS

SEQ ID NO: 116 - protein, 13 aa, Homo sapiens
WVSAISYNSANIY

SEQ ID NO: 117 - protein, 11 aa, Homo sapiens
ARRLGWGNGFD

SEQ ID NO: 118 - protein, 119 aa, Homo sapiens; identical to SEQ ID NO: 114

SEQ ID NO: 119 - protein, 6 aa, Homo sapiens
SSYSMS

SEQ ID NO: 120 - protein, 13 aa, Homo sapiens
WVSAISYNSANIY

SEQ ID NO: 121 - protein, 11 aa, Homo sapiens
ARRLGWGNGFD

SEQ ID NO: 122 - protein, 119 aa, Homo sapiens
EVQLLESGGGLVQPGGSLRLSCAASGFTFSSYAMSWVRQAPGKGLEWVSVISYSGAYIYYADSVKGRFTISRDNSKNTLYLQMNSLRAEDTAVYYCARKVGWGHGMDYWGQGTLVTVSS

SEQ ID NO: 123 - protein, 6 aa, Homo sapiens
SSYAMS

SEQ ID NO: 124 - protein, 13 aa, Homo sapiens
WVSVISYSGAYIY

SEQ ID NO: 125 - protein, 11 aa, Homo sapiens
ARKVGWGHGMD

SEQ ID NO: 126 - protein, 119 aa, Homo sapiens
EVQLLESGGGLVQPGGSLRLSCAASGFTFSSYAMSWVRQAPGKGLEWVASISNGGTITNYADSVKGRFTISRDNSKNTLYLQMNSLRAEDTAVYYCARGYASSRGFDYWGQGTLVTVSS

SEQ ID NO: 127 - protein, 6 aa, Homo sapiens
SSYAMS

SEQ ID NO: 128 - protein, 13 aa, Homo sapiens
WVASISNGGTITN

SEQ ID NO: 129 - protein, 11 aa, Homo sapiens
ARGYASSRGFD

SEQ ID NO: 130 - protein, 120 aa, Homo sapiens
EVQLVESGGGLVKPGGSLRLSCAASGFTFSDYGMHWVRQAPGKGLEWVARISNNGAIIYYADSVKGRFTISRDNAKNSLYLQMNSLRAEDTAVYYCARGGYGGYYAFDYWGQGTLVTVSS

SEQ ID NO: 131 - protein, 6 aa, Homo sapiens
SDYGMH

SEQ ID NO: 132 - protein, 13 aa, Homo sapiens
WVARISNNGAIIY

SEQ ID NO: 133 - protein, 12 aa, Homo sapiens
ARGGYGGYYAFD

SEQ ID NO: 134 - protein, 120 aa, Homo sapiens
QVQLVQSGAEVKKPGASVKVSCKASGYTFSNYYMHWVRQAPGQGLEWMGGINPINGTAKYAQKFQGRVTMTRDTSISTAYMELSRLRSDDTAVYYCARRGYGGYYTFDYWGQGTLVTVSS

SEQ ID NO: 135 - protein, 6 aa, Homo sapiens
SNYYMH

SEQ ID NO: 136 - protein, 13 aa, Homo sapiens
WMGGINPINGTAK

SEQ ID NO: 137 - protein, 12 aa, Homo sapiens
ARRGYGGYYTFD

SEQ ID NO: 138 - protein, 120 aa, Homo sapiens
EVQLLESGGGLVQPGGSLRLSCAASGFTFRNYSMSWVRQAPGKGLEWVAGIGWDSAIKYYADSVKGRFTISRDNSKNTLYLQMNSLRAEDTAVYYCARGTSGGRDAFDYWGQGTLVTVSS

SEQ ID NO: 139 - protein, 6 aa, Homo sapiens
RNYSMS

SEQ ID NO: 140 - protein, 13 aa, Homo sapiens
WVAGIGWDSAIKY

SEQ ID NO: 141 - protein, 12 aa, Homo sapiens
ARGTSGGRDAFD

SEQ ID NO: 142 - protein, 120 aa, Homo sapiens
EVQLVESGGGLVKPGGSLRLSCAASGFTFSDYGMHWVRQAPGKGLEWVARISNNGAIIYYADSVKGRFTISRDNAKNSLYLQMNSLRAEDTAVYYCARGGTSGYYAFDYWGQGTLVTVSS

SEQ ID NO: 143 - protein, 6 aa, Homo sapiens
SDYGMH

SEQ ID NO: 144 - protein, 13 aa, Homo sapiens
WVARISNNGAIIY

SEQ ID NO: 145 - protein, 12 aa, Homo sapiens
ARGGTSGYYAFD

SEQ ID NO: 146 - protein, 120 aa, Homo sapiens
EVQLLESGGGLVQPGGSLRLSCAASGFTFSSYAMSWVRQAPGKGLEWVSSISYNGGNKYYADSVKGRFTISRDNSKNTLYLQMNSLRAEDTAVYYCARGQWGYRAPFDYWGQGTLVTVSS

SEQ ID NO: 147 - protein, 6 aa, Homo sapiens
SSYAMS

SEQ ID NO: 148 - protein, 13 aa, Homo sapiens
WVSSISYNGGNKY

SEQ ID NO: 149 - protein, 12 aa, Homo sapiens
ARGQWGYRAPFD

SEQ ID NO: 150 - protein, 120 aa, Homo sapiens
EVQLLESGGGLVQPGGSLRLSCAASGFTFRNYSMSWVRQAPGKGLEWVASISAGSAYKNYADSVKGRFTISRDNSKNTLYLQMNSLRAEDTAVYYCARGLWSAGYAFDYGGQGTLVTVSS

SEQ ID NO: 151 - protein, 6 aa, Homo sapiens
RNYSMS

SEQ ID NO: 152 - protein, 13 aa, Homo sapiens
WVASISAGSAYKN

SEQ ID NO: 153 - protein, 12 aa, Homo sapiens
ARGLWSAGYAFD

SEQ ID NO: 154 - protein, 120 aa, Homo sapiens
EVQLLESGGGLVQPGGSLRLSCAASGFTFRSFSMSWVRQAPGKGLEWVAAISYNSANTYYADSVKGRFTISRDNSKNTLYLQMNSLRAEDTAVYYCARRAAWSRSPFDYWGQGTLVTVSS

SEQ ID NO: 155 - protein, 6 aa, Homo sapiens
RSFSMS

SEQ ID NO: 156 - protein, 13 aa, Homo sapiens
WVAAISYNSANTY

SEQ ID NO: 157 - protein, 12 aa, Homo sapiens
ARRAAWSRSPFD

SEQ ID NO: 158 - protein, 120 aa, Homo sapiens
QVQLVQSGAEVKKPGASVKVSCKASGYTFTGYYMHWVRQAPGQGLEWMGSINPFNGSTNYAQKFQGRVTMTRDTSISTAYMELSRLRSDDTAVYYCARRGWWTSSAFDYWGQGTLVTVSS

SEQ ID NO: 159 - protein, 6 aa, Homo sapiens
TGYYMH

SEQ ID NO: 160 - protein, 13 aa, Homo sapiens
WMGSINPFNGSTN

SEQ ID NO: 161 - protein, 12 aa, Homo sapiens
ARRGWWTSSAFD

SEQ ID NO: 162 - protein, 120 aa, Homo sapiens
EVQLVESGGGLVKPGGSLRLSCAASGFTFRSYAMSWVRQAPGKGLEWVASINSNGAYTNYADSVKGRFTISRDNAKNSLYLQMNSLRAEDTAVYYCARGRGAYDRGFDYWGQGTLVTVSS

SEQ ID NO: 163 - protein, 6 aa, Homo sapiens
RSYAMS

SEQ ID NO: 164 - protein, 13 aa, Homo sapiens
WVASINSNGAYTN

SEQ ID NO: 165 - protein, 12 aa, Homo sapiens
ARGRGAYDRGFD

SEQ ID NO: 166 - protein, 120 aa, Homo sapiens
EVQLLESGGGLVQPGGSLRLSCAASGFTFSTYAMHWVRQAPGKGLEWVAGISGGGTYKYYADSVKGRFTISRDNSKNTLYLQMNSLRAEDTAVYYCARPRSVAYANFDYWGQGTLVTVSS

SEQ ID NO: 167 - protein, 6 aa, Homo sapiens
STYAMH

SEQ ID NO: 168 - protein, 13 aa, Homo sapiens
WVAGISGGGTYKY

SEQ ID NO: 169 - protein, 12 aa, Homo sapiens
ARPRSVAYANFD

SEQ ID NO: 170 - protein, 120 aa, Homo sapiens
EVQLLESGGGLVQPGGSLRLSCAASGFTFSNYSMHWVRQAPGKGLEWVAGIWGDSGYIYYADSVKGRFTISRDNSKNTLYLQMNSLRAEDTAVYYCARARVLAADGFDYWGQGTLVTVSS

SEQ ID NO: 171 - protein, 6 aa, Homo sapiens
SNYSMH

SEQ ID NO: 172 - protein, 13 aa, Homo sapiens
WVAGIWGDSGYIY

SEQ ID NO: 173 - protein, 12 aa, Homo sapiens
ARARVLAADGFD

SEQ ID NO: 174 - protein, 121 aa, Homo sapiens
EVQLVESGGGLVKPGGSLRLSCAASGFTFRNYGMNWVRQAPGKGLEWVAGIKNDGDTKYYADSVKGRFTISRDNAKNSLYLQMNSLRAEDTAVYYCAKGRYKGYVGPLDYWGQGTLVTVSS

SEQ ID NO: 175 - protein, 6 aa, Homo sapiens
RNYGMN

SEQ ID NO: 176 - protein, 13 aa, Homo sapiens
WVAGIKNDGDTKY

SEQ ID NO: 177 - protein, 13 aa, Homo sapiens
AKGRYKGYVGPLD

SEQ ID NO: 178 - protein, 121 aa, Homo sapiens
EVQLVESGGGLVKPGGSLRLSCAASGFTFRNYGMSWVRQAPGKGLEWVAGIWSNSGIINYADSVKGRFTISRDNAKNSLYLQMNSLRAEDTAVYYCAKSSYASYWSAFDYWGQGTLVTVSS

SEQ ID NO: 179 - protein, 6 aa, Homo sapiens
RNYGMS

SEQ ID NO: 180 - protein, 13 aa, Homo sapiens
WVAGIWSNSGIIN

SEQ ID NO: 181 - protein, 13 aa, Homo sapiens
AKSSYASYWSAFD

SEQ ID NO: 182 - protein, 121 aa, Homo sapiens
EVQLVESGGGLVKPGGSLRLSCAASGFTFINYAMSWVRQAPGKGLEWVASIGNDSTNTYYADSVKGRFTISRDNAKNSLYLQMNSLRAENTAVYYCAKSRYIALSRPLDYWGQGTLVTVSS

SEQ ID NO: 183 - protein, 6 aa, Homo sapiens
INYAMS

SEQ ID NO: 184 - protein, 13 aa, Homo sapiens
WVASIGNDSTNTY

SEQ ID NO: 185 - protein, 13 aa, Homo sapiens
AKSRYIALSRPLD

SEQ ID NO: 186 - protein, 122 aa, Homo sapiens
EVQLVESGGGLVKPGGSLRLSCAASGFTFSSYSMNWVRQAPGKGLEWVSSISSSSSYIYYADSVKGRFTISRDNAKNSLYLQMNSLRAEDTAVYYCARGPRPSYYAGWFDYWGQGTLVTVSS

SEQ ID NO: 187 - protein, 6 aa, Homo sapiens
SSYSMN

SEQ ID NO: 188 - protein, 13 aa, Homo sapiens
WVSSISSSSSYIY

SEQ ID NO: 189 - protein, 14 aa, Homo sapiens
ARGPRPSYYAGWFD

SEQ ID NO: 190 - protein, 122 aa, Homo sapiens
EVQLVESGGGLVKPGGSLRLSCAASGFTFSNYSMSWVRQAPGKGLEWVSGISGGGAYKYYADSVKGRFTISRDNAKNSLYLQMNSLRAEDTAVYYCARAGSRSPRYYHFDYWGQGTLVTVSS

SEQ ID NO: 191 - protein, 6 aa, Homo sapiens
SNYSMS

SEQ ID NO: 192 - protein, 13 aa, Homo sapiens
WVSGISGGGAYKY

SEQ ID NO: 193 - protein, 14 aa, Homo sapiens
ARAGSRSPRYYHFD

SEQ ID NO: 194 - protein, 121 aa, Homo sapiens
QVQLLESGGDLVHPGGSLRRSGAHRGFTFMSNAWSGVLQAPGKGRKGGVGFSRGPGNITYPNSSKGPFPFPRDNSNPLNWKMNSLRAENTAFYYCARVARTYEMHYGFDYGGQGTLVTVSS

SEQ ID NO: 195 - protein, 6 aa, Homo sapiens
MSNAWS

SEQ ID NO: 196 - protein, 15 aa, Homo sapiens
GGVGFSRGPGNITRV

SEQ ID NO: 197 - protein, 12 aa, Homo sapiens
ARTYEMHYGFDY

SEQ ID NO: 198 - protein, 122 aa, Homo sapiens
EVQLLESGGGLVQPGGSLRLSCAASGFTFSSYAMSWVRQAPGKGLEWVAGISGGSGNISYADSVKGRFTISRDNSKNTLYLQMNSLRAEDTAVYYCARVARSYERDYGFDYWGQGTLVTVSS

SEQ ID NO: 199 - protein, 6 aa, Homo sapiens
SSYAMS

SEQ ID NO: 200 - protein, 16 aa, Homo sapiens
WVAGISGGSGNISARV

SEQ ID NO: 201 - protein, 11 aa, Homo sapiens
ARSYERDYGFD

SEQ ID NO: 202 - protein, 122 aa, Homo sapiens
EVQLVESGGGLVKPGGSLRLSCAASGFTFSNYGMHWVRQAPGKGLEWVARISGGGGYTYYADSVKGRFTISRDNAKNSLYLQMNSLRAEDTAVYYCAREDSLGGGNYYFDYWGQGTLVTVSS

SEQ ID NO: 203 - protein, 6 aa, Homo sapiens
SNYGMH

SEQ ID NO: 204 - protein, 13 aa, Homo sapiens
WVARISGGGGYTY

SEQ ID NO: 205 - protein, 14 aa, Homo sapiens
AREDSLGGGNYYFD

SEQ ID NO: 206 - protein, 123 aa, Homo sapiens
EVQLVESGGGLVKPGGSLRLSCAASGFTFSSYGMSWVRQAPGKGLEWVAGINSSGRNKYYADSVKGRFTISRDNAKNSLYLQMNSLRAEDTAVYYCARGFYAVRSDVGAMDYWGQGTLVTVSS

SEQ ID NO: 207 - protein, 6 aa, Homo sapiens
SSYGMS

SEQ ID NO: 208 - protein, 13 aa, Homo sapiens
WVAGINSSGRNKY

SEQ ID NO: 209 - protein, 15 aa, Homo sapiens
ARGFYAVRSDVGAMD

SEQ ID NO: 210 - protein, 123 aa, Homo sapiens
EVQLVESGGGLVKPGGSLRLSCAASGFTFSNYGMHWVRQAPGKGLEWVSSISSSSSYIYYADSVKGRFTISRDNAKNSLYLQMNSLRAEDTAVYYCARAFNAWRGNESNGDYWGQGTLVTVSS

SEQ ID NO: 211 - protein, 6 aa, Homo sapiens
SNYGMH

SEQ ID NO: 212 - protein, 13 aa, Homo sapiens
WVSSISSSSSYIY

SEQ ID NO: 213 - protein, 15 aa, Homo sapiens
ARAFNAWRGNESNGD

SEQ ID NO: 214 - protein, 121 aa, Homo sapiens
EVQLVESGGGLVKPGGSLRLSCAASGFTFRTYGMHWVRQAPGKGLEWVAGINYSGNNKYYADSVKGRFTISRDNAKNSLYLQMNSLRAEDTAVYYCARDSSTTRTRALDYWGQGTLVTVSS

SEQ ID NO: 215 - protein, 6 aa, Homo sapiens
RTYGMH

SEQ ID NO: 216 - protein, 13 aa, Homo sapiens
WVAGINYSGNNKY

SEQ ID NO: 217 - protein, 13 aa, Homo sapiens
ARDSSTTRTRALD

SEQ ID NO: 218 - protein, 121 aa, Homo sapiens
EVQLVESGGGLVKPGGSLRLSCAASGFTFRSYGMHWVRQAPGKGLEWVAGINYSGNNKYYADSVKGRFTISRDNAKNSLYLQMNSLRAEDTAVYYCARDSSTTRTRALDYWGQGTLVTVSS

SEQ ID NO: 219 - protein, 6 aa, Homo sapiens
RSYGMH

SEQ ID NO: 220 - protein, 13 aa, Homo sapiens
WVAGINYSGNNKY

SEQ ID NO: 221 - protein, 13 aa, Homo sapiens
ARDSSTTRTRALD

SEQ ID NO: 222 - protein, 121 aa, Homo sapiens
EVQLVESGGGLVKPGGSLRLSCAASGFTFSSFGMHWVRQAPGKGLEWVAGINYSGNNKYYADSVKGRFTISRDNAKNSLYLQMNSLRAEDTAVYYCARDSSTTRTRALDYWGQGTLVTVSS

SEQ ID NO: 223 - protein, 6 aa, Homo sapiens
SSFGMH

SEQ ID NO: 224 - protein, 13 aa, Homo sapiens
WVAGINYSGNNKY

SEQ ID NO: 225 - protein, 13 aa, Homo sapiens
ARDSSTTRTRALD

SEQ ID NO: 226 - protein, 121 aa, Homo sapiens
EVQLVESGGGLVKPGGSLRLSCAASGFTFSTYGMHWVRQAPGKGLEWVSGINYSGNNKYYADSVKGRFTISRDNAKNSLYLQMNSLRAEDTAVYYCARDSSTTRTRALDYWGQGTLVTVSS

SEQ ID NO: 227 - protein, 6 aa, Homo sapiens
STYGMH

SEQ ID NO: 228 - protein, 13 aa, Homo sapiens
WVSGINYSGNNKY

SEQ ID NO: 229 - protein, 13 aa, Homo sapiens
ARDSSTTRTRALD

SEQ ID NO: 230 - protein, 121 aa, Homo sapiens
EVQLVESGGGLVKPGGSLRLSCAASGFTFSNYGMHWVRQAPGKGLEWVAGINYSGNNKYYADSVKGRFTISRDNAKNSLYLQMNSLRAEDTAVYYCARDSSTTRTRALDYWGQGTLVTVSS

SEQ ID NO: 231 - protein, 6 aa, Homo sapiens
SNYGMH

SEQ ID NO: 232 - protein, 13 aa, Homo sapiens
WVAGINYSGNNKY

SEQ ID NO: 233 - protein, 13 aa, Homo sapiens
ARDSSTTRTRALD

SEQ ID NO: 234 - protein, 121 aa, Homo sapiens
EVQLVESGGGLVKPGGSLRLSCAASGFTFSSYGMHWVRQAPGKGLEWVAGINYSGNNKYYADSVKGRFTISRDNAKNSLYLQMNSLRAEDTAVYYCARDSSTTRTRALDYWGQGTLVTVSS

SEQ ID NO: 235 - protein, 6 aa, Homo sapiens
SSYGMH

SEQ ID NO: 236 - protein, 13 aa, Homo sapiens
WVAGINYSGNNKY

SEQ ID NO: 237 - protein, 13 aa, Homo sapiens
ARDSSTTRTRALD

SEQ ID NO: 238 - protein, 121 aa, Homo sapiens
EVQLVESGGGLVKPGGSLRLSCAASGFTFRSFGMHWVRQAPGKGLEWVAGINYSGNNKYYADSVKGRFTISRDNAKNSLYLQMNSLRAEDTAVYYCARDSSTTRTRALDYWGQGTLVTVSS

SEQ ID NO: 239 - protein, 6 aa, Homo sapiens
RSFGMH

SEQ ID NO: 240 - protein, 13 aa, Homo sapiens
WVAGINYSGNNKY

SEQ ID NO: 241 - protein, 13 aa, Homo sapiens
ARDSSTTRTRALD

SEQ ID NO: 242 - protein, 121 aa, Homo sapiens
EVQLVESGGGLVKPGGSLRLSCAASGFTFSSYGMHWVRQAPGKGLEWVAGINFSGNNKYYADSVKGRFTISRDNAKNSLYLQMNSLRAEDTAVYYCARDSSTTRTRALDYWGQGTLVTVSS

SEQ ID NO: 243 - protein, 6 aa, Homo sapiens
SSYGMH

SEQ ID NO: 244 - protein, 13 aa, Homo sapiens
WVAGINFSGNNKY

SEQ ID NO: 245 - protein, 13 aa, Homo sapiens
ARDSSTTRTRALD

SEQ ID NO: 246 - protein, 121 aa, Homo sapiens
EVQLVESGGGLVKPGGSLRLSCAASGFTFSSYGMHWVRQAPGKGLEWVTGINYSGNNRYYADSVKGRFTISRDNAKNSLYLQMNSLRAEDTAVYYCARDSSTTRTRALDYWGQGTLVTVSS

SEQ ID NO: 247 - protein, 6 aa, Homo sapiens
SSYGMH

SEQ ID NO: 248 - protein, 13 aa, Homo sapiens
WVTGINYSGNNRY

SEQ ID NO: 249 - protein, 13 aa, Homo sapiens
ARDSSTTRTRALD

SEQ ID NO: 250 - protein, 121 aa, Homo sapiens
EVQLVESGGGLVKPGGSLRLSCAASGFTFSDYGMHWVRQAPGKGLEWVAGNNYSGNNKYYADSVKGRFTISRDNAKNSLYLQMNSLRAEDTAVYYCARDSSTTRTRALDYWGQGTLVTVSS

SEQ ID NO: 251 - protein, 6 aa, Homo sapiens
SDYGMH

SEQ ID NO: 252 - protein, 13 aa, Homo sapiens
WVAGNNYSGNNKY

SEQ ID NO: 253 - protein, 13 aa, Homo sapiens
ARDSSTTRTRALD

SEQ ID NO: 254 - protein, 121 aa, Homo sapiens
EVQLVESGGGLVKPGGSLRLSCAASGFTFSDYGMHWVRQAPGKGLEWVAGINYSGNNRYYADSVKGRFTISRDNAKNSLYLQMNSLRAEDTAVYYCARDSSTTRTRALDYWGQGTLVTVSS

SEQ ID NO: 255 - protein, 6 aa, Homo sapiens
SDYGMH

SEQ ID NO: 256 - protein, 13 aa, Homo sapiens
WVAGINYSGNNKY

SEQ ID NO: 257 - protein, 13 aa, Homo sapiens
ARDSSTTRTRALD

SEQ ID NO: 258 - protein, 121 aa, Homo sapiens
EVQLVESGGGLVKPGGSLRLSCAASGFTFRSFGMHWVRQAPGKGLEWVAGINYSGNNRYYADSVKGRFTISRDNAKNSLYLQMNSLRAEDTAVYYCARDSSTVRTRALDYWGQGTLVTVSS

SEQ ID NO: 259 - protein, 6 aa, Homo sapiens
RSFGMH

SEQ ID NO: 260 - protein, 13 aa, Homo sapiens
WVAGINYSGNNKY

SEQ ID NO: 261 - protein, 13 aa, Homo sapiens
ARDSSTVRTRALD

SEQ ID NO: 262 - protein, 121 aa, Homo sapiens
EVQLVESGGGLVKPGGSLRLSCAASGFTFRSFGMHWVRQAPGKGLEWVAGINYSGNNRYYADSVKGRFTISRDNAKNSLYLQMNSLRAEDTAVYYCARDSSTTRTRSLDYWGQGTLVTVSS

SEQ ID NO: 263 - protein, 6 aa, Homo sapiens
RSFGMH

SEQ ID NO: 264 - protein, 13 aa, Homo sapiens
WVAGINYSGNNKY

SEQ ID NO: 265 - protein, 13 aa, Homo sapiens
ARDSSTVRTRSLD

SEQ ID NO: 266 - protein, 121 aa, Homo sapiens
EVQLVESGGGLVKPGGSLRLSCAASGFTFRSFGMHWVRQAPGKGLEWVAGINYSGNNRYYADSVKGRFTISRDNAKNSLYLQMNSLRAEDTAVYYCARDSSTIRTRSLDYWGQGTLVTVSS

SEQ ID NO: 267 - protein, 6 aa, Homo sapiens
RSFGMH

SEQ ID NO: 268 - protein, 13 aa, Homo sapiens
WVAGINYSGNNKY

SEQ ID NO: 269 - protein, 13 aa, Homo sapiens
ARDSSTIRTRSLD

SEQ ID NO: 270 - protein, 121 aa, Homo sapiens
EVQLVESGGGLVKPGGSLRLSCAASGFTFSTYGMHWVRQAPGKGLEWVSGINYSGNNIYYADSVKGRFTISRDNAKNSLYLQMNSLRAEDTAVYYCARDSSTTRTRSLDYWGQGTLVTVSS

SEQ ID NO: 271 - protein, 6 aa, Homo sapiens
STYGMH

SEQ ID NO: 272 - protein, 13 aa, Homo sapiens
WVSGINYSGNNIY

SEQ ID NO: 273 - protein, 13 aa, Homo sapiens
ARDSSTTRTRSLD

SEQ ID NO: 274 - protein, 121 aa, Homo sapiens
EVQLVESGGGLVKPGGSLRLSCAASGFTFSTYGMHWVRQAPGKGLEWVAGINYSGNNIYYADSVKGRFTISRDNAKNSLYLQMNSLRAEDTAVYYCARDSSTTRTRSLDYWGQGTLVTVSS

SEQ ID NO: 275 - protein, 6 aa, Homo sapiens
STYGMH

SEQ ID NO: 276 - protein, 13 aa, Homo sapiens
WVAGINYSGNNIY

SEQ ID NO: 277 - protein, 13 aa, Homo sapiens
ARDSSTTRTRSLD

SEQ ID NO: 278 - protein, 121 aa, Homo sapiens
EVQLVESGGGLVKPGGSLRLSCAASGFTFSDYGMHWVRQAPGKGLEWVAGVNYSGNNIYYADSVKGRFTISRDNAKNSLYLQMNSLRAEDTAVYYCARDSSTTRTRSLDYWGQGTLVTVSS

SEQ ID NO: 279 - protein, 6 aa, Homo sapiens
SDYGMH

SEQ ID NO: 280 - protein, 13 aa, Homo sapiens
WVAGVNYSGNNIY

SEQ ID NO: 281 - protein, 13 aa, Homo sapiens
ARDSSTTRTRSLD

SEQ ID NO: 282 - protein, 121 aa, Homo sapiens
EVQLVESGGGLVKPGGSLRLSCAASGFTFRSFGMHWVRQAPGKGLEWVAGVNYSGNNIYYADSVKGRFTISRDNAKNSLYLQMNSLRAEDTAVYYCARDSSTNRGRSLDYWGQGTLVTVSS

SEQ ID NO: 283 - protein, 6 aa, Homo sapiens
RSFGMH

SEQ ID NO: 284 - protein, 13 aa, Homo sapiens
WVAGVNYSGNNIY

SEQ ID NO: 285 - protein, 13 aa, Homo sapiens
ARDSSTNRGRSLD

SEQ ID NO: 286 - protein, 121 aa, Homo sapiens
EVQLVESGGGLVKPGGSLRLSCAASGFTFRSFGMHWVRQAPGKGLEWVAGVNYSGNNIYYADSVKGRFTISRDNAKNSLYLQMNSLRAEDTAVYYCARDRSSIRGRPLDYWGQGTLVTVSS

SEQ ID NO: 287 - protein, 6 aa, Homo sapiens
RSFGMH

SEQ ID NO: 288 - protein, 13 aa, Homo sapiens
WVAGVNYSGNNIY

SEQ ID NO: 289 - protein, 13 aa, Homo sapiens
ARDRSSIRGRPLD

SEQ ID NO: 290 - protein, 121 aa, Homo sapiens
EVQLVESGGGLVKPGGSLRLSCAASGFTFSNFGMHWVRQAPGKGLEWVAAISYSGSYTYYADSVKGRFTISRDNAKNSLYLQMNSLRAEDTAVYYCARDSSAVRGRPLDYWGQGTLVTVSS

SEQ ID NO: 291 - protein, 6 aa, Homo sapiens
SNFGMH

SEQ ID NO: 292 - protein, 13 aa, Homo sapiens
WVAAISYSGSYTY

SEQ ID NO: 293 - protein, 13 aa, Homo sapiens
ARDSSAVRGRPLD

SEQ ID NO: 294 - protein, 121 aa, Homo sapiens
EVQLVESGGGLVKPGGSLRLSCAASGFTFSTYGMHWVRQAPGKGLEWVAGINYSGNNKYYADSVKGRFTISRDNAKNSLYLQMNSLRAEDTAVYYCARDSSTNRTRALDYWGQGTLVTVSS

SEQ ID NO: 295 - protein, 6 aa, Homo sapiens
STYGMH

SEQ ID NO: 296 - protein, 13 aa, Homo sapiens
WVAGINYSGNNKY

SEQ ID NO: 297 - protein, 13 aa, Homo sapiens
ARDSSTNRTRALD

SEQ ID NO: 298 - protein, 121 aa, Homo sapiens
EVQLVESGGGLVKPGGSLRLSCAASGFTFSTYGMHWVRQAPGKGLEWVAGINYSGNNKYYADSVKGRFTISRDNAKNSLYLQMNSLRAEDTAVYYCARDSSTNLTRSLDYWGQGTLVTVSS

SEQ ID NO: 299 - protein, 6 aa, Homo sapiens
STYGMH

SEQ ID NO: 300 - protein, 13 aa, Homo sapiens
WVAGINYSGNNKY

SEQ ID NO: 301 - protein, 13 aa, Homo sapiens
ARDSSTNLTRSLD

SEQ ID NO: 302 - protein, 121 aa, Homo sapiens
EVQLVESGGGLVKPGGSLRLSCAASGFTFSTYGMHWVRQAPGKGLEWVAGINYSGNNKYYADSVKGRFTISRDNAKNSLYLQMNSLRAEDTAVYYCARDSSTNLTRTLDYWGQGTLVTVSS

SEQ ID NO: 303 - protein, 6 aa, Homo sapiens
STYGMH

SEQ ID NO: 304 - protein, 13 aa, Homo sapiens
WVAGINYSGNNKY

SEQ ID NO: 305 - protein, 13 aa, Homo sapiens
ARDSSTNLTRTLD

SEQ ID NO: 306 - protein, 121 aa, Homo sapiens
EVQLVESGGGLVKPGGSLRLSCAASGFTFSTYGMHWVRQAPGKGLEWVAGINYSGNNKYYADSVKGRFTISRDNAKNSLYLQMNSLRAEDTAVYYCARDSSTNLTRALDYWGQGTLVTVSS

SEQ ID NO: 307 - protein, 6 aa, Homo sapiens
STYGMH

SEQ ID NO: 308 - protein, 13 aa, Homo sapiens
WVAGINYSGNNKY

SEQ ID NO: 309 - protein, 13 aa, Homo sapiens
ARDSSTNLTRALD

SEQ ID NO: 310 - protein, 121 aa, Homo sapiens; identical to SEQ ID NO: 294

SEQ ID NO: 311 - protein, 6 aa, Homo sapiens
STYGMH

SEQ ID NO: 312 - protein, 13 aa, Homo sapiens
WVAGINYSGNNKY

SEQ ID NO: 313 - protein, 13 aa, Homo sapiens
ARDSSTNRTRALD

SEQ ID NO: 314 - protein, 121 aa, Homo sapiens
EVQLVESGGGLVKPGGSLRLSCAASGFTFSTYGMHWVRQAPGKGLEWVAGINYSGNNKYYADSVKGRFTISRDNAKNSLYLQMNSLRAEDTAVYYCARDSSTNWTRALDYWGQGTLVTVSS

SEQ ID NO: 315 - protein, 6 aa, Homo sapiens
STYGMH

SEQ ID NO: 316 - protein, 13 aa, Homo sapiens
WVAGINYSGNNKY

SEQ ID NO: 317 - protein, 13 aa, Homo sapiens
ARDSSTNWTRALD

SEQ ID NO: 318 - protein, 121 aa, Homo sapiens
EVQLVESGGGLVKPGGSLRLSCAASGFTFSTYGMHWVRQAPGKGLEWVAGINYSGNNKYYADSVKGRFTISRDNAKNSLYLQMNSLRAEDTAVYYCARDSSTNYTRALDYWGQGTLVTVSS

SEQ ID NO: 319 - protein, 6 aa, Homo sapiens
STYGMH

SEQ ID NO: 320 - protein, 13 aa, Homo sapiens
WVAGINYSGNNKY

SEQ ID NO: 321 - protein, 13 aa, Homo sapiens
ARDSSTNYTRALD

SEQ ID NO: 322 - protein, 121 aa, Homo sapiens
EVQLVESGGGLVKPGGSLRLSCAASGFTFSTYGMHWVRQAPGKGLEWVAGINYSGNNKYYADSVKGRFTISRDNAKNSLYLQMNSLRAEDTAVYYCARDHSSNRSRSLDYWGQGTLVTVSS

SEQ ID NO: 323 - protein, 6 aa, Homo sapiens
STYGMH

SEQ ID NO: 324 - protein, 13 aa, Homo sapiens
WVAGINYSGNNKY

SEQ ID NO: 325 - protein, 13 aa, Homo sapiens
ARDHSSNRSRSLD

SEQ ID NO: 326 - protein, 121 aa, Homo sapiens
EVQLVESGGGLVKPGGSLRLSCAASGFTFSTYGMHWVRQAPGKGLEWVAGINYSGNNKYYADSVKGRFTISRDNAKNSLYLQMNSLRAEDTAVYYCARDHSSNVSRSLDYWGQGTLVTVSS

SEQ ID NO: 327 - protein, 6 aa, Homo sapiens
STYGMH

SEQ ID NO: 328 - protein, 13 aa, Homo sapiens
WVAGINYSGNNKY

SEQ ID NO: 329 - protein, 13 aa, Homo sapiens
ARDHSSNVSRSLD

SEQ ID NO: 330 - protein, 121 aa, Homo sapiens
EVQLVESGGGLVKPGGSLRLSCAASGFTFSTYGMHWVRQAPGKGLEWVAGINYSGNNKYYADSVKGRFTISRDNAKNSLYLQMNSLRAEDTAVYYCARDHSSNRSRDLDYWGQGTLVTVSS

SEQ ID NO: 331 - protein, 6 aa, Homo sapiens
STYGMH

SEQ ID NO: 332 - protein, 13 aa, Homo sapiens
WVAGINYSGNNKY

SEQ ID NO: 333 - protein, 13 aa, Homo sapiens
ARDHSSNRSRDLD

SEQ ID NO: 334 - protein, 121 aa, Homo sapiens
EVQLVESGGGLVKPGGSLRLSCAASGFTFSTYGMHWVRQAPGKGLEWVAGINYSGNNKYYADSVKGRFTISRDNAKNSLYLQMNSLRAEDTAVYYCARDHSSNFSRHLDYWGQGTLVTVSS

SEQ ID NO: 335 - protein, 6 aa, Homo sapiens
STYGMH

SEQ ID NO: 336 - protein, 13 aa, Homo sapiens
WVAGINYSGNNKY

SEQ ID NO: 337 - protein, 13 aa, Homo sapiens
ARDHSSNFSRHLD

SEQ ID NO: 338 - protein, 121 aa, Homo sapiens
EVQLVESGGGLVKPGGSLRLSCAASGFTFSTYGMHWVRQAPGKGLEWVAGINYSGNNKYYADSVKGRFTISRDNAKNSLYLQMNSLRAEDTAVYYCARDHSSTRGRSLDYWGQGTLVTVSS

SEQ ID NO: 339 - protein, 6 aa, Homo sapiens
STYGMH

SEQ ID NO: 340 - protein, 13 aa, Homo sapiens
WVAGINYSGNNKY

SEQ ID NO: 341 - protein, 13 aa, Homo sapiens
ARDHSSTRGRSLD

SEQ ID NO: 342 - protein, 121 aa, Homo sapiens
EVQLVESGGGLVKPGGSLRLSCAASGFTFSTYGMHWVRQAPGKGLEWVAGINYSGNNKYYADSVKGRFTISRDNAKNSLYLQMNSLRAEDTAVYYCARDHSSTRSRSLDYWGQGTLVTVSS

SEQ ID NO: 343 - protein, 6 aa, Homo sapiens
STYGMH

SEQ ID NO: 344 - protein, 13 aa, Homo sapiens
WVAGINYSGNNKY

SEQ ID NO: 345 - protein, 13 aa, Homo sapiens
ARDHSSTRSRSLD

SEQ ID NO: 346 - protein, 121 aa, Homo sapiens
EVQLVESGGGLVKPGGSLRLSCAASGFTFSTYGMHWVRQAPGKGLEWVAGINYSGNNKYYADSVKGRFTISRDNAKNSLYLQMNSLRAEDTAVYYCARDHSSTWSRSLDYWGQGTLVTVSS

SEQ ID NO: 347 - protein, 6 aa, Homo sapiens
STYGMH

SEQ ID NO: 348 - protein, 13 aa, Homo sapiens
WVAGINYSGNNKY

SEQ ID NO: 349 - protein, 13 aa, Homo sapiens
ARDHSSTWSRSLD

SEQ ID NO: 350 - protein, 121 aa, Homo sapiens
EVQLVESGGGLVKPGGSLRLSCAASGFTFSTYGMHWVRQAPGKGLEWVAGINYSGNNKYYADSVKGRFTISRDNAKNSLYLQMNSLRAEDTAVYYCARDHSSNRGRSLDYWGQGTLVTVSS

SEQ ID NO: 351 - protein, 6 aa, Homo sapiens
STYGMH

SEQ ID NO: 352 - protein, 13 aa, Homo sapiens
WVAGINYSGNNKY

SEQ ID NO: 353 - protein, 13 aa, Homo sapiens
ARDHSSNRGRSLD

SEQ ID NO: 354 - protein, 121 aa, Homo sapiens
EVQLVESGGGLVKPGGSLRLSCAASGFTFSTYGMHWVRQAPGKGLEWVAGINYSGNNKYYADSVKGRFTISRDNAKNSLYLQMNSLRAEDTAVYYCARDHSSTLYRALDYWGQGTLVTVSS

SEQ ID NO: 355 - protein, 6 aa, Homo sapiens
STYGMH

SEQ ID NO: 356 - protein, 13 aa, Homo sapiens
WVAGINYSGNNKY

SEQ ID NO: 357 - protein, 13 aa, Homo sapiens
ARDHSSTLYRALD

SEQ ID NO: 358 - protein, 121 aa, Homo sapiens
EVQLVESGGGLVKPGGSLRLSCAASGFTFSTYGMHWVRQAPGKGLEWVAGINYSGNNKYYADSVKGRFTISRDNAKNSLYLQMNSLRAEDTAVYYCARDHSSTLHRALDYWGQGTLVTVSS

SEQ ID NO: 359 - protein, 6 aa, Homo sapiens
STYGMH

SEQ ID NO: 360 - protein, 13 aa, Homo sapiens
WVAGINYSGNNKY

SEQ ID NO: 361 - protein, 13 aa, Homo sapiens
ARDHSSTLHRALD

SEQ ID NO: 362 - protein, 121 aa, Homo sapiens
EVQLVESGGGLVKPGGSLRLSCAASGFTFSTYGMHWVRQAPGKGLEWVAGINYSGNNKYYADSVKGRFTISRDNAKNSLYLQMNSLRAEDTAVYYCARDHSSNLYRALDYWGQGTLVTVSS

SEQ ID NO: 363 - protein, 6 aa, Homo sapiens
STYGMH

SEQ ID NO: 364 - protein, 13 aa, Homo sapiens
WVAGINYSGNNKY

SEQ ID NO: 365 - protein, 13 aa, Homo sapiens
ARDHSSNLYRALD

SEQ ID NO: 366 - protein, 121 aa, Homo sapiens
EVQLVESGGGLVKPGGSLRLSCAASGFTFSTYGMHWVRQAPGKGLEWVAGINYSGNNKYYADSVKGRFTISRDNAKNSLYLQMNSLRAEDTAVYYCARDHSGYWTRSLDYWGQGTLVTVSS

SEQ ID NO: 367 - protein, 6 aa, Homo sapiens
STYGMH

SEQ ID NO: 368 - protein, 13 aa, Homo sapiens
WVAGINYSGNNKY

SEQ ID NO: 369 - protein, 13 aa, Homo sapiens
ARDHSGYWTRSLD

SEQ ID NO: 370 - protein, 121 aa, Homo sapiens
EVQLVESGGGLVKPGGSLRLSCAASGFTFSTYGMHWVRQAPGKGLEWVAGINYSGNNKYYADSVKGRFTISRDNAKNSLYLQMNSLRAEDTAVYYCARDRSNIVGRPLDYWGQGTLVTVSS

SEQ ID NO: 371 - protein, 6 aa, Homo sapiens
STYGMH

SEQ ID NO: 372 - protein, 13 aa, Homo sapiens
WVAGINYSGNNKY

SEQ ID NO: 373 - protein, 13 aa, Homo sapiens
ARDRSNIVGRPLD

SEQ ID NO: 374 - protein, 121 aa, Homo sapiens
EVQLVESGGGLVKPGGSLRLSCAASGFTFSTYGMHWVRQAPGKGLEWVAGINYSGNNKYYADSVKGRFTISRDNAKNSLYLQMNSLRAEDTAVYYCARDRSSIRGRPLDYWGQGTLVTVSS

SEQ ID NO: 375 - protein, 6 aa, Homo sapiens
STYGMH

SEQ ID NO: 376 - protein, 13 aa, Homo sapiens
WVAGINYSGNNKY

SEQ ID NO: 377 - protein, 13 aa, Homo sapiens
ARDRSSIRGRPLD

SEQ ID NO: 378 - protein, 121 aa, Homo sapiens
EVQLVESGGGLVKPGGSLRLSCAASGFTFSTYGMHWVRQAPGKGLEWVAGINYSGNNKYYADSVKGRFTISRDNAKNSLYLQMNSLRAEDTAVYYCARDRSTTYSRALDYWGQGTLVTVSS

SEQ ID NO: 379 - protein, 6 aa, Homo sapiens
STYGMH

SEQ ID NO: 380 - protein, 13 aa, Homo sapiens
WVAGINYSGNNKY

SEQ ID NO: 381 - protein, 13 aa, Homo sapiens
ARDRSTTYSRALD

SEQ ID NO: 382 - protein, 121 aa, Homo sapiens
EVQLVESGGGLVKPGGSLRLSCAASGFTFSTYGMHWVRQAPGKGLEWVAGINYSGNNKYYADSVKGRFTISRDNAKNSLYLQMNSLRAEDTAVYYCARDRSTTLNRALDYWGQGTLVTVSS

SEQ ID NO: 383 - protein, 6 aa, Homo sapiens
STYGMH

SEQ ID NO: 384 - protein, 13 aa, Homo sapiens
WVAGINYSGNNKY

SEQ ID NO: 385 - protein, 13 aa, Homo sapiens
ARDRSTTLNRALD

SEQ ID NO: 386 - protein, 121 aa, Homo sapiens
EVQLVESGGGLVKPGGSLRLSCAASGFTFSTYGMHWVRQAPGKGLEWVAGINYSGNNKYYADSVKGRFTISRDNAKNSLYLQMNSLRAEDTAVYYCARDHSTNRGRSLDYWGQGTLVTVSS

SEQ ID NO: 387 - protein, 6 aa, Homo sapiens
STYGMH

SEQ ID NO: 388 - protein, 13 aa, Homo sapiens
WVAGINYSGNNKY

SEQ ID NO: 389 - protein, 13 aa, Homo sapiens
ARDHSTNRGRSLD

SEQ ID NO: 390 - protein, 121 aa, Homo sapiens
EVQLVESGGGLVKPGGSLRLSCAASGFTFSTYGMHWVRQAPGKGLEWVAGINYSGNNKYYADSVKGRFTISRDNAKNSLYLQMNSLRAEDTAVYYCARDHSTNLGRSLDYWGQGTLVTVSS

SEQ ID NO: 391 - protein, 6 aa, Homo sapiens
STYGMH

SEQ ID NO: 392 - protein, 13 aa, Homo sapiens
WVAGINYSGNNKY

SEQ ID NO: 393 - protein, 13 aa, Homo sapiens
ARDHSTNLGRSLD

SEQ ID NO: 394 - protein, 121 aa, Homo sapiens
  VARIANT 107: Xaa=any amino
EVQLVESGGGLVKPGGSLRLSCAASGFTFSTYGMHWVRQAPGKGLEWVAGINYSGNNKYYADSVKGRFTISRDNAKNSLYLQMNSLRAEDTAVYYCARDHSTNRRRXLDYWGQGTLVTVSS

SEQ ID NO: 395 - protein, 6 aa, Homo sapiens
STYGMH

SEQ ID NO: 396 - protein, 13 aa, Homo sapiens
WVAGINYSGNNKY

SEQ ID NO: 397 - protein, 13 aa, Homo sapiens
  VARIANT 11: Xaa=any amino
ARDHSTNRRRXLD

SEQ ID NO: 398 - protein, 121 aa, Homo sapiens
EVQLVESGGGLVKPGGSLRLSCAASGFTFSTYGMHWVRQAPGKGLEWVAGINYSGNNKYYADSVKGRFTISRDNAKNSLYLQMNSLRAEDTAVYYCARDSSTNRSRSLDYWGQGTLVTVSS

SEQ ID NO: 399 - protein, 6 aa, Homo sapiens
STYGMH

SEQ ID NO: 400 - protein, 13 aa, Homo sapiens
WVAGINYSGNNKY

SEQ ID NO: 401 - protein, 13 aa, Homo sapiens
ARDSSTNRSRSLD

SEQ ID NO: 402 - protein, 121 aa, Homo sapiens
EVQLVESGGGLVKPGGSLRLSCAASGFTFSTYGMHWVRQAPGKGLEWVAGINYSGNNKYYADSVKGRFTISRDNAKNSLYLQMNSLRAEDTAVYYCARDSSTTRSRTLDYWGQGTLVTVSS

SEQ ID NO: 403 - protein, 6 aa, Homo sapiens
STYGMH

SEQ ID NO: 404 - protein, 13 aa, Homo sapiens
WVAGINYSGNNKY

SEQ ID NO: 405 - protein, 13 aa, Homo sapiens
ARDSSTTRSRTLD

SEQ ID NO: 406 - protein, 121 aa, Homo sapiens
EVQLVESGGGLVKPGGSLRLSCAASGFTFSTYGMHWVRQAPGKGLEWVAGINYSGNNKYYADSVKGRFTISRDNAKNSLYLQMNSLRAEDTAVYYCARDSSTTRSRSLDYWGQGTLVTVSS

SEQ ID NO: 407 - protein, 6 aa, Homo sapiens
STYGMH

SEQ ID NO: 408 - protein, 13 aa, Homo sapiens
WVAGINYSGNNKY

SEQ ID NO: 409 - protein, 13 aa, Homo sapiens
ARDSSTTRSRSLD

SEQ ID NO: 410 - protein, 121 aa, Homo sapiens
EVQLVESGGGLVKPGGSLRLSCAASGFTFSTYGMHWVRQAPGKGLEWVAGINYSGNNKYYADSVKGRFTISRDNAKNSLYLQMNSLRAEDTAVYYCARDSSTNRSRALDYWGQGTLVTVSS

SEQ ID NO: 411 - protein, 6 aa, Homo sapiens
STYGMH

SEQ ID NO: 412 - protein, 13 aa, Homo sapiens
WVAGINYSGNNKY

SEQ ID NO: 413 - protein, 13 aa, Homo sapiens
ARDSSTNRSRALD

SEQ ID NO: 414 - protein, 121 aa, Homo sapiens
EVQLVESGGGLVKPGGSLRLSCAASGFTFSTYGMHWVRQAPGKGLEWVAGINYSGNNKYYADSVKGRFTISRDNAKNSLYLQMNSLRAEDTAVYYCARDSSTNRGRALDYWGQGTLVTVSS

SEQ ID NO: 415 - protein, 6 aa, Homo sapiens
STYGMH

SEQ ID NO: 416 - protein, 13 aa, Homo sapiens
WVAGINYSGNNKY

SEQ ID NO: 417 - protein, 13 aa, Homo sapiens
ARDSSTNRGRALD

SEQ ID NO: 418 - protein, 121 aa, Homo sapiens
EVQLVESGGGLVKPGGSLRLSCAASGFTFSTYGMHWVRQAPGKGLEWVAGINYSGNNKYYADSVKGRFTISRDNAKNSLYLQMNSLRAEDTAVYYCARDSSTVRGRALDYWGQGTLVTVSS

SEQ ID NO: 419 - protein, 6 aa, Homo sapiens
STYGMH

SEQ ID NO: 420 - protein, 13 aa, Homo sapiens
WVAGINYSGNNKY

SEQ ID NO: 421 - protein, 13 aa, Homo sapiens
ARDSSTVRGRALD

SEQ ID NO: 422 - protein, 121 aa, Homo sapiens
EVQLVESGGGLVKPGGSLRLSCAASGFTFSTYGMHWVRQAPGKGLEWVAGINYSGNNKYYADSVKGRFTISRDNAKNSLYLQMNSLRAEDTAVYYCARDSSTNRTRSLDYWGQGTLVTVSS

SEQ ID NO: 423 - protein, 6 aa, Homo sapiens
STYGMH

SEQ ID NO: 424 - protein, 13 aa, Homo sapiens
WVAGINYSGNNKY

SEQ ID NO: 425 - protein, 13 aa, Homo sapiens
ARDSSTNRTRSLD

SEQ ID NO: 426 - protein, 121 aa, Homo sapiens
EVQLVESGGGLVKPGGSLRLSCAASGFTFSTYGMHWVRQAPGKGLEWVAGINYSGNNKYYADSVKGRFTISRDNAKNSLYLQMNSLRAEDTAVYYCARDSSTNRTRSLDYWGRGTLVTVSS

SEQ ID NO: 427 - protein, 6 aa, Homo sapiens
STYGMH

SEQ ID NO: 428 - protein, 13 aa, Homo sapiens
WVAGINYSGNNKY

SEQ ID NO: 429 - protein, 13 aa, Homo sapiens
ARDSSTNRTRSLD

SEQ ID NO: 430 - protein, 121 aa, Homo sapiens
EVQLVESGGGLVKPGGSLRLSCAASGFTFSTYGMHWVRQAPGKGLEWVAGINYSGNNKYYADSVKGRFTISRDNAKNSLYLQMNSLRAEDTAVYYCARDSSTVRTRSLDYWGQGTLVTVSS

SEQ ID NO: 431 - protein, 6 aa, Homo sapiens
STYGMH

SEQ ID NO: 432 - protein, 13 aa, Homo sapiens
WVAGINYSGNNKY

SEQ ID NO: 433 - protein, 13 aa, Homo sapiens
ARDSSTVRTRSLD

SEQ ID NO: 434 - protein, 121 aa, Homo sapiens
EVQLVESGGGLVKPGGSLRLSCAASGFTFSTYGMHWVRQAPGKGLEWVAGINYSGNNKYYADSVKGRFTISRDNAKNSLYLQMNSLRAEDTAVYYCARDSSTTRTRSLDYWGQGTLVTVSS

SEQ ID NO: 435 - protein, 6 aa, Homo sapiens
STYGMH

SEQ ID NO: 436 - protein, 13 aa, Homo sapiens
WVAGINYSGNNKY

SEQ ID NO: 437 - protein, 13 aa, Homo sapiens
ARDSSTTRTRSLD

SEQ ID NO: 438 - protein, 121 aa, Homo sapiens
EVQLVESGGGLVKPGGSLRLSCAASGFTFSTYGMHWVRQAPGKGLEWVAGINYSGNNKYYADSVKGRFTISRDNAKNSLYLQMNSLRAEDTAVYYCARDTSTNRTRGLDYWGQGTLVTVSS

SEQ ID NO: 439 - protein, 6 aa, Homo sapiens
STYGMH

SEQ ID NO: 440 - protein, 13 aa, Homo sapiens
WVAGINYSGNNKY

SEQ ID NO: 441 - protein, 13 aa, Homo sapiens
ARDTSTNRTRGLD

SEQ ID NO: 442 - protein, 121 aa, Homo sapiens
EVQLVESGGGLVKPGGSLRLSCAASGFTFSTYGMHWVRQAPGKGLEWVAGINYSGNNKYYADSVKGRFTISRDNAKNSLYLQMNSLRAEDTAVYYCARDSSTNRTRGLDYWGQGTLVTVSS

SEQ ID NO: 443 - protein, 6 aa, Homo sapiens
STYGMH

SEQ ID NO: 444 - protein, 13 aa, Homo sapiens
WVAGINYSGNNKY

SEQ ID NO: 445 - protein, 13 aa, Homo sapiens
ARDSSTNRTRGLD

SEQ ID NO: 446 - protein, 121 aa, Homo sapiens
EVQLVESGGGLVKPGGSLRLSCAASGFTFSTYGMHWVRQAPGKGLEWVAGINYSGNNKYYADSVKGRFTISRDNAKNSLYLQMNSLRAEDTAVYYCARDSSTIRTRGLDYWGQGTLVTVSS

SEQ ID NO: 447 - protein, 6 aa, Homo sapiens
STYGMH

SEQ ID NO: 448 - protein, 13 aa, Homo sapiens
WVAGINYSGNNKY

SEQ ID NO: 449 - protein, 13 aa, Homo sapiens
ARDSSTIRTRGLD

SEQ ID NO: 450 - protein, 121 aa, Homo sapiens
EVQLVESGGGLVKPGGSLRLSCAASGFTFSTYGMHWVRQAPGKGLEWVAGINYSGNNKYYADSVKGRFTISRDNAKNSLYLQMNSLRAEDTAVYYCARDSSTTRTRGLDYWGQGTLVTVSS

SEQ ID NO: 451 - protein, 6 aa, Homo sapiens
STYGMH

SEQ ID NO: 452 - protein, 13 aa, Homo sapiens
WVAGINYSGNNKY

SEQ ID NO: 453 - protein, 13 aa, Homo sapiens
ARDSSTTRTRGLD

SEQ ID NO: 454 - protein, 121 aa, Homo sapiens
EVQLVESGGGLVKPGGSLRLSCAASGFTFSTYGMHWVRQAPGKGLEWVAGINYSGNNKYYADSVKGRFTISRDNAKNSLYLQMNSLRAEDTAVYYCARDSSTNRTRTLDYWGQGTLVTVSS

SEQ ID NO: 455 - protein, 6 aa, Homo sapiens
STYGMH

SEQ ID NO: 456 - protein, 13 aa, Homo sapiens
WVAGINYSGNNKY

SEQ ID NO: 457 - protein, 13 aa, Homo sapiens
ARDSSTNRTRTLD

SEQ ID NO: 458 - protein, 121 aa, Homo sapiens
EVQLVESGGGLVKPGGSLRLSCAASGFTFSTYGMHWVRQAPGKGLEWVAGINYSGNNKYYADSVKGRFTISRDNAKNSLYLQMNSLRAEDTAVYYCARDSSTTRTRALDYWGQGTLVTVSS

SEQ ID NO: 459 - protein, 6 aa, Homo sapiens
STYGMH

SEQ ID NO: 460 - protein, 13 aa, Homo sapiens
WVAGINYSGNNKY

SEQ ID NO: 461 - protein, 13 aa, Homo sapiens
ARDSSTTRTRALD

SEQ ID NO: 462 - protein, 121 aa, Homo sapiens
EVQLVESGGGLVKPGGSLRLSCAASGFTFSTYGMHWVRQAPGKGLEWVAGINYSGNNKYYADSVKGRFTISRDNAKNSLYLQMNSLRAEDTAVYYCARDSSTVRTRALDYWGQGTLVTVSS

SEQ ID NO: 463 - protein, 6 aa, Homo sapiens
STYGMH

SEQ ID NO: 464 - protein, 13 aa, Homo sapiens
WVAGINYSGNNKY

SEQ ID NO: 465 - protein, 13 aa, Homo sapiens
ARDSSTVRTRALD

SEQ ID NO: 466 - protein, 121 aa, Homo sapiens
EVQLVESGGGLVKPGGSLRLSCAASGFTFSTYGMHWVRQAPGKGLEWVAGINYSGNNKYYADSVKGRFTISRDNAKNSLYLQMNSLRAEDTAVYYCARDSSTISTRALDYWGQGTLVTVSS

SEQ ID NO: 467 - protein, 6 aa, Homo sapiens
STYGMH

SEQ ID NO: 468 - protein, 13 aa, Homo sapiens
WVAGINYSGNNKY

SEQ ID NO: 469 - protein, 13 aa, Homo sapiens
ARDSSTISTRALD

SEQ ID NO: 470 - protein, 121 aa, Homo sapiens
EVQLVESGGGLVKPGGSLRLSCAASGFTFSTYGMHWVRQAPGKGLEWVAGINYSGNNKYYADSVKGRFTISRDNAKNSLYLQMNSLRAEDTAVYYCARDSSTIRTRALDYWGQGTLVTVSS

SEQ ID NO: 471 - protein, 6 aa, Homo sapiens
STYGMH

SEQ ID NO: 472 - protein, 13 aa, Homo sapiens
WVAGINYSGNNKY

SEQ ID NO: 473 - protein, 13 aa, Homo sapiens
ARDSSTIRTRALD

SEQ ID NO: 474 - protein, 467 aa, Homo sapiens
APPPARVHLGAFLAVTPNPGSAASGTEAAAATPSKVWGSSAGRIEPRGGGRGALPTSMGQHGPSARARAGRAPGPRPAREASPRLRVHKTFKFVVVGVLLQVVPSSAATIKLHDQSIGTQQWEHSPLGELCPPGSHRSEHPGACNRCTEGVGYTNASNNLFACLPCTACKSDEEERSPCTTTRNTACQCKPGTFRNDNSAEMCRKCSRGCPRGMVKVKDCTPWSDIECVHKESGNGHNIWVILVVTLVVPLLLVAVLIVCCCIGSGCGGDPKCMDRVCFWRLGLLRGPGAEDNAHNEILSNADSLSTFVSEQQMESQEPADLTGVTVQSPGEAQCLLGPAEAEGSQRRRLLVPANGADPTETLMLFFDKFANIVPFDSWDQLMRQLDLTKNEIDVVRAGTAGPGDALYAMLMKWVNKTGRNASIHTLLDALERMEERHAKEKIQDLLVDSGKFIYLEDGTGSAVSLE

SEQ ID NO: 475 - protein, 468 aa, Homo sapiens [sequence omitted]

SEQ ID NO: 476 - protein, 468 aa, Homo sapiens
MAPPPARVHLGAFLAVTPNPGSAASGTEAAAATPSKVWGSSAGRIEPRGGGRGALPTSMGQHGPSARARAGRAPGPRPAREASPRLRVHKTFKFVVVGVLLQVVPSSAATIKLHDQSIGTQQWEHSPLGELCPPGSHRSERPGACNRCTEGVGYTNASNNLFACLPCTACKSDEEERSPCTTTRNTACQCKPGTFRNDNSAEMCRKCSTGCPRGMVKVKDCTPWSDIECVHKESGNGHNIWVILVVTLVVPLLLVAVLIVCCCIGSGCGGDPKCMDRVCFWRLGLLRGPGAEDNAHNEILSNADSLSTFVSEQQMESQEPADLTGVTVQSPGEAQCLLGPAEAEGSQRRRLLVPANGADPTETLMLFFDKFANIVPFDSWDQLMRQLDLTKNEIDVVRAGTAGPGDALYAMLMKWVNKTGRNASIHTLLDALERMEERHAKEKIQDLLVDSGKFIYLEDGTGSAVSLE

SEQ ID NO: 477 - protein, 468 aa, Homo sapiens; identical to SEQ ID NO: 476

SEQ ID NO: 478 - protein, 448 aa, Homo sapiens
MEQRGQNAPAASGARKRHGPGPREARGARPGPRVPKTLVLVVAAVLLLVSAESALITQQDLAPQQRAAPQQKRSSPSEGLCPPGHHISEDGRDCISCKYGQDYSTHWNDLLFCLRCTRCDSGEVELSPCTTTRNTVCQCEEGTFREEDSPEMCRKCRTGCPRGMVKVGDCTPWSDIECVHKESGTKHSGEAPAVEETVTSSPGTPASPCSLSGIIIGVTVAAVVLIVAVFVCKSLLWKKVLPYLKGICBIVALENTSBPGGDPERVDRSSQRPGAEDNVLNEIVSILQPTQVPEQEMEVQEPAEPTGVNMLSPGESEHLLEPAEAERSQRRRLLVPANEGDPTETLRQCFDDFADLVPFDSWEPLMRKLGLMDNEIKVAKAEAAGHRDTLYTMLIKWVNKTGRDASVHTLLDALETLGERLAKQKIEDHLLSSGKFMYLEGNADSAMS

SEQ ID NO: 479 - protein, 448 aa, Homo sapiens
MEQRGQNAPAASGARKRHGPGPREARGARPGPRVPKTLVLVVAAVLLLVSAESALITQQDLAPQQRAAPQQKRSSPSEGLCPPGHHISEDGRDCISCKYGQDYSTHWNDLLFCLRCTRCDSGEVELSPCTTTRNTVCQCEEGTFREEDSPEMCRKCRTGCPRGMVKVGDCTPWSDIECVHKESGTKHSGEVPAVEETVTSSPGTPASPCSLSGIIIGVTVAAVVLIVAVFVCKSLLWKKVLPYLKGICBIVALENTSBPGGDPERVDRSSQRPGAEDNVLNEIVSILQPTQVPEQEMEVQEPAEPTGVNMLSPGESEHLLEPAEAERSQRRRLLVPANEGDPTETLRQCFDDFADLVPFDSWEPLMRKLGLMDNEIKVAKAEAAGHRDTLYTMLIKWVNKTGRDASVHTLLDALETLGERLAKQKIEDHLLSSGKFMYLEGNADSAMS

SEQ ID NO: 480 - protein, 448 aa, Homo sapiens
MEQRGQNAPAASGARKRHGPGPREARGARPGLRVPKTLVLVVAAVLLLVSAESALITQQDLAPQQRAAPQQKRSSPSEGLCPPGHHISEDGRDCISCKYGQDYSTHWNDLLFCLRCTRCDSGEVELSPCTTTRNTVCQCEEGTFREEDSPEMCRKCRTGCPRGMVKVGDCTPWSDIECVHKESGTKHSGEAPAVEETVTSSPGTPASPCSLSGIIIGVTVAAVVLIVAVFVCKSLLWKKVLPYLKGICBIVALENTSBPGGDPERVDRSSQRPGAEDNVLNEIVSILQPTQVPEQEMEVQEPAEPTGVNMLSPGESEHLLEPAEAERSQRRRLLVPANEGDPTETLRQCFDDFADLVPFDSWEPLMRKLGLMDNEIKVAKAEAAGHRDTLYTMLIKWVNKTGRDASVHTLLDALETLGERLAKQKIEDHLLSSGKFMYLEGNADSAMS

SEQ ID NO: 481 - protein, 448 aa, Homo sapiens
MEQRGQNAPAASGARKRHGPGPREARGARPGLRVPKTLVLVVAAVLLLVSAESALITQQDLAPQQRVAPQQKRSSPSEGLCPPGHHISEDGRDCISCKYGQDYSTHWNDLLFCLRCTRCDSGEVELSPCTTTRNTVCQCEEGTFREEDSPEMCRKCRTGCPRGMVKVGDCTPWSDIECVHKESGTKHSGEAPAVEETVTSSPGTPASPCSLSGIIIGVTVAAVVLIVAVFVCKSLLWKKVLPYLKGICBIVALENTSBPGGDPERVDRSSQRPGAEDNVLNEIVSILQPTQVPEQEMEVQEPAEPTGVNMLSPGESEHLLEPAEAERSQRRRLLVPANEGDPTETLRQCFDDFADLVPFDSWEPLMRKLGLMDNEIKVAKAEAAGHRDTLYTMLIKWVNKTGRDASVHTLLDALETLGERLAKQKIEDHLLSSGKFMYLEGNADSAMS

SEQ ID NO: 482 - protein, 448 aa, Homo sapiens
MEQRGQNAPAASGARKRHGPGPREAWGARPGLRVPKTLVLVVAAVLLLVSAESALITQQDLAPQQRVAPQQKRSSPSEGLCPPGHHISEDGRDCISCKYGQDYSTHWNDLLFCLRCTRCDSGEVELSPCTTTRNTVCQCEEGTFREEDSPEMCRKCRTGCPRGMVKVGDCTPWSDIECVHKESGTKHSGEAPAVEETVTSSPGTPASPCSLSGIIIGVTVAAVVLIVAVFVCKSLLWKKVLPYLKGICBIVALENTSBPGGDPERVDRSSQRPGAEDNVLNEIVSILQPTQVPEQEMEVQEPAEPTGVNMLSPGESEHLLEPAEAERSQRRRLLVPANEGDPTETLRQCFDDFADLVPFDSWEPLMRKLGLMDNEIKVAKAEAAGHRDTLYTMLIKWVNKTGRDASVHTLLDALETLGERLAKQKIEDHLLSSGKFMYLEGNADSAMS

SEQ ID NO: 483 - protein, 223 aa, Artificial Sequence
  Synthetic Construct
QPVLHQPPAMSSALGTTIRLTCTLRNDHDIGVYSVYWYQQRPGHPPRFLLRYFSQSDKSQGPQVPPRFSGSKDVARNRGYLSISELQPEDEAMYYCAMGARSSVTHVFGSGTQLTVLSQPKATPSVTLFPPSSEELQANKATLVCLMNDFYPGILTVTWKADGTPITQGVEMTTPSKQSNNKYAASSYLSLTPEQWRSRRSYSCQVMHEGSTVEKTVAPAECS

SEQ ID NO: 484 - protein, 10 aa, Homo sapiens
  VARIANT (1)...(1): Xaa = D or E
  VARIANT (2)...(2): Xaa = I, V or L
  VARIANT (3)...(3): Xaa = G or A
  VARIANT 4, 7: Xaa = V, I or L
  VARIANT 5, 8, 10: Xaa = Y or F
  VARIANT (6)...(6): Xaa = S or T
XXXXXXXXWX

SEQ ID NO: 485 - protein, 13 aa, Homo sapiens
  VARIANT 1, 2: Xaa = L, I or V
  VARIANT (3)...(3): Xaa = R or K
  VARIANT (4)...(4): Xaa = Y or F
  VARIANT (5)...(5): Xaa = F or Y
  VARIANT 6, 8, 11: Xaa = S or T
  VARIANT 7, 12: Xaa = Q or N
  VARIANT (9)...(9): Xaa = D or E
  VARIANT (10)...(10): Xaa = K or R
  VARIANT (13)...(13): Xaa = G or A
XXXXXXXXXXXXX

SEQ ID NO: 486 - protein, 10 aa, Homo sapiens
  VARIANT 1, 4: Xaa = A or G
  VARIANT (2)...(2): Xaa = M or L
  VARIANT (3)...(3): Xaa = G or A
  VARIANT (4)...(4): Xaa = A or G
  VARIANT (5)...(5): Xaa = R or K
  VARIANT 6, 7: Xaa = S or T
  VARIANT (8)...(8): Xaa = V, I or L
  VARIANT (9)...(9): Xaa = T or S
XXXXXXXXXH

SEQ ID NO: 487 - protein, 223 aa, Artificial Sequence
  Synthetic Construct
QPVLHQPPAMSSALGCTIRLTCTLRNDHDIGVYSVYWYQQRPGHPPRFLLRYFSQSDKSQGPQVPPRFSGSKDVARNRGYLSISELQPEDEAMYYCAMGARSSVTHVFGSGTQLTVLSQPKATPSVTLFPPSSEELQANKATLVCLMNDFYPGILTVTWKADGTPITQGVEMTTPSKQSNNKYAASSYLSLTPEQWRSRRSYSCQVMHEGSTVEKTVAPAECS

SEQ ID NO: 488 - protein, 223 aa, Artificial Sequence
  Synthetic Construct
QPVLHQPPAMSSALGTTIRLCCTLRNDHDIGVYSVYWYQQRPGHPPRFLLRYFSQSDKSQGPQVPPRFSGSKDVARNRGYLSISELQPEDEAMYYCAMGARSSVTHVFGSGTQLTVLSQPKATPSVTLFPPSSEELQANKATLVCLMNDFYPGILTVTWKADGTPITQGVEMTTPSKQSNNKYAASSYLSLTPEQWRSRRSYSCQVMHEGSTVEKTVAPAECS

SEQ ID NO: 489 - protein, 223 aa, Artificial Sequence
  Synthetic Construct
QPVLHQPPAMSSALGTTIRLTCTLRNDHDIGVYSVYWYQQRPGHPPRFLLRYFSQSDKSQGPQVPPRFSGSKDVARNRGYLSISELQPEDEAMYYCAMGARSSVTHCFGSGTQLTVLSQPKATPSVTLFPPSSEELQANKATLVCLMNDFYPGILTVTWKADGTPITQGVEMTTPSKQSNNKYAASSYLSLTPEQWRSRRSYSCQVMHEGSTVEKTVAPAECS

SEQ ID NO: 490 - protein, 223 aa, Artificial Sequence
  Synthetic Construct
QPVLHQPPAMSSALGTTIRLTCTLRNDHDIGVYSVYWYQQRPGHPPRFLLRYFSQSDKSQGPQVPPRFSGSKDVARNRGYLSISELQPEDEAMYYCAMGARSSVTHVFGSGTQLTVLSQPCATPSVTLFPPSSEELQANKATLVCLMNDFYPGILTVTWKADGTPITQGVEMTTPSKQSNNKYAASSYLSLTPEQWRSRRSYSCQVMHEGSTVEKTVAPAECS

SEQ ID NO: 491 - protein, 223 aa, Artificial Sequence
  Synthetic Construct
QPVLHQPPAMSSALGTTIRLTCTLRNDHDIGVYSVYWYQQRPGHPPRFLLRYFSQSDKSQGPQVPPRFSGSKDVARNRGYLSISELQPEDEAMYYCAMGARSSVTHVFGSGTQLTVLSQPKATPCVTLFPPSSEELQANKATLVCLMNDFYPGILTVTWKADGTPITQGVEMTTPSKQSNNKYAASSYLSLTPEQWRSRRSYSCQVMHEGSTVEKTVAPAECS

SEQ ID NO: 492 - protein, 223 aa, Artificial Sequence
  Synthetic Construct
QPVLHQPPAMSSALGTTIRLTCTLRNDHDIGVYSVYWYQQRPGHPPRFLLRYFSQSDKSQGPQVPPRFSGSKDVARNRGYLSISELQPEDEAMYYCAMGARSSVTHVFGSGTQLTVLSQPKATPSCTLFPPSSEELQANKATLVCLMNDFYPGILTVTWKADGTPITQGVEMTTPSKQSNNKYAASSYLSLTPEQWRSRRSYSCQVMHEGSTVEKTVAPAECS

SEQ ID NO: 493 - protein, 223 aa, Artificial Sequence
  Synthetic Construct
QPVLHQPPAMSSALGTTIRLTCTLRNDHDIGVYSVYWYQQRPGHPPRFLLRYFSQSDKSQGPQVPPRFSGSKDVARNRGYLSISELQPEDEAMYYCAMGARSSVTHVFGSGTQLTVLSQPKATPSVTLFPPCSEELQANKATLVCLMNDFYPGILTVTWKADGTPITQGVEMTTPSKQSNNKYAASSYLSLTPEQWRSRRSYSCQVMHEGSTVEKTVAPAECS

SEQ ID NO: 494 - protein, 223 aa, Artificial Sequence
  Synthetic Construct
QPVLHQPPAMSSALGTTIRLTCTLRNDHDIGVYSVYWYQQRPGHPPRFLLRYFSQSDKSQGPQVPPRFSGSKDVARNRGYLSISELQPEDEAMYYCAMGARSSVTHVFGSGTQLTVLSQPKATPSVTLFPPSSEELQCNKATLVCLMNDFYPGILTVTWKADGTPITQGVEMTTPSKQSNNKYAASSYLSLTPEQWRSRRSYSCQVMHEGSTVEKTVAPAECS

SEQ ID NO: 495 - protein, 223 aa, Artificial Sequence
  Synthetic Construct
QPVLHQPPAMSSALGTTIRLTCTLRNDHDIGVYSVYWYQQRPGHPPRFLLRYFSQSDKSQGPQVPPRFSGSKDVARNRGYLSISELQPEDEAMYYCAMGARSSVTHVFGSGTQLTVLSQPKATPSVTLFPPSSEELQANKATLVCLMNDFYPGILTCTWKADGTPITQGVEMTTPSKQSNNKYAASSYLSLTPEQWRSRRSYSCQVMHEGSTVEKTVAPAECS

SEQ ID NO: 496 - protein, 223 aa, Artificial Sequence
  Synthetic Construct
QPVLHQPPAMSSALGTTIRLTCTLRNDHDIGVYSVYWYQQRPGHPPRFLLRYFSQSDKSQGPQVPPRFSGSKDVARNRGYLSISELQPEDEAMYYCAMGARSSVTHVFGSGTQLTVLSQPKATPSVTLFPPSSEELQANKATLVCLMNDFYPGILTVTWKADGTPITQGCEMTTPSKQSNNKYAASSYLSLTPEQWRSRRSYSCQVMHEGSTVEKTVAPAECS

SEQ ID NO: 497 - protein, 223 aa, Artificial Sequence
  Synthetic Construct
QPVLHQPPAMSSALGTTIRLTCTLRNDHDIGVYSVYWYQQRPGHPPRFLLRYFSQSDKSQGPQVPPRFSGSKDVARNRGYLSISELQPEDEAMYYCAMGARSSVTHVFGSGTQLTVLSQPKATPSVTLFPPSSEELQANKATLVCLMNDFYPGILTVTWKADGTPITQGVEMTTPSKCSNNKYAASSYLSLTPEQWRSRRSYSCQVMHEGSTVEKTVAPAECS

SEQ ID NO: 498 - protein, 223 aa, Artificial Sequence
  Synthetic Construct
QPVLHQPPAMSSALGTTIRLTCTLRNDHDIGVYSVYWYQQRPGHPPRFLLRYFSQSDKSQGPQVPPRFSGSKDVARNRGYLSISELQPEDEAMYYCAMGARSSVTHVFGSGTQLTVLSQPKATPSVTLFPPSSEELQANKATLVCLMNDFYPGILTVTWKADGTPITQGVEMTTPSKQSCNKYAASSYLSLTPEQWRSRRSYSCQVMHEGSTVEKTVAPAECS

SEQ ID NO: 499 - protein, 223 aa, Artificial Sequence
  Synthetic Construct
QPVLHQPPAMSSALGTTIRLTCTLRNDHDIGVYSVYWYQQRPGHPPRFLLRYFSQSDKSQGPQVPPRFSGSKDVARNRGYLSISELQPEDEAMYYCAMGARSSVTHVFGSGTQLTVLSQPKATPSVTLFPPSSEELQANKATLVCLMNDFYPGILTVTWKADGTPITQGVEMTTPSKQSNNKYAASSYLSLTPEQWRSRRSYSCQVMHEGSTCEKTVAPAECS

SEQ ID NO: 500 - protein, 223 aa, Artificial Sequence
  Synthetic Construct
QPVLHQPPAMSSALGTTIRLTCTLRNDHDIGVYSVYWYQQRPGHPPRFLLRYFSQSDKSQGPQVPPRFSGSKDVARNRGYLSISELQPEDEAMYYCAMGARSSVTHVFGSGTQLTVLSQPKATPSVTLFPPSSEELQANKATLVCLMNDFYPGILTVTWKADGTPITQGVEMTTPSKQSNNKYAASSYLSLTPEQWRSRRSYSCQVMHEGSTVEKTCAPAECS

SEQ ID NO: 501 - protein, 121 aa, Artificial Sequence
  Synthetic Construct
GSQSVLTQPPSVSAAPGQKVTISCSGSSSNIGNNYVSWYQQLPGTAPKLLIYDNNKRPSGIPDRFSGSKSGTSATLGITGLQTGDEADYYCGTWDSSLSAVVFGGGTKLTVLRTASGAAAA